European Patent Application EP 4 413 993 A1, published August 14, 2024. Title: METHOD OF OBTAINING RECOMBINANT HUMAN BRAIN-DERIVED NEUROTROPHIC FACTOR. Applicant: Dompé Farmaceutici. The sequence listing filed with the application follows.

SEQUENCE LISTING (22 sequences)

SEQ ID NO: 1 - protein, 119 aa, Homo sapiens
HSDPARRGELSVCDSISEWVTAADKKTAVDMSGGTVTVLEKVPVSKGQLKQYFYETKCNPMGYTKEGCRGIDKRHWNSQCRTTQSYVRALTMDSKKRIGWRFIRIDTSCVCTLTIKRGR

SEQ ID NO: 2 - protein, 229 aa, Homo sapiens
APMKEANIRGQGGLAYPGVRTHGTLESVNGPKAGSRGLTSLADTFEHVIEELLDEDQKVRPNEENNKDADLYTSRVMLSSQVPLEPPLLFLLEEYKNYLDAANMSMRVRRHSDPARRGELSVCDSISEWVTAADKKTAVDMSGGTVTVLEKVPVSKGQLKQYFYETKCNPMGYTKEGCRGIDKRHWNSQCRTTQSYVRALTMDSKKRIGWRFIRIDTSCVCTLTIKRGR

SEQ ID NO: 3 - protein, 230 aa, synthetic construct
  VARIANT 108..110: note = selected from non-basic amino acids and histidine
  VARIANT 111: note = Arginine or Lysine
MAPMKEANIRGQGGLAYPGVRTHGTLESVNGPKAGSRGLTSLADTFEHVIEELLDEDQKVRPNEENNKDADLYTSRVMLSSQVPLEPPLLFLLEEYKNYLDAANMSMXXXXHSDPARRGELSVCDSISEWVTAADKKTAVDMSGGTVTVLEKVPVSKGQLKQYFYETKCNPMGYTKEGCRGIDKRHWNSQCRTTQSYVRALTMDSKKRIGWRFIRIDTSCVCTLTIKRGR

SEQ ID NO: 4 - protein, 230 aa, synthetic construct
MAPMKEANIRGQGGLAYPGVRTHGTLESVNGPKAGSRGLTSLADTFEHVIEELLDEDQKVRPNEENNKDADLYTSRVMLSSQVPLEPPLLFLLEEYKNYLDAANMSMVSARHSDPARRGELSVCDSISEWVTAADKKTAVDMSGGTVTVLEKVPVSKGQLKQYFYETKCNPMGYTKEGCRGIDKRHWNSQCRTTQSYVRALTMDSKKRIGWRFIRIDTSCVCTLTIKRGR

SEQ ID NO: 5 - protein, 230 aa, synthetic construct; identical to SEQ ID NO: 3
  VARIANT 108..110: note = selected from the group consisting of Alanine, Asparagine, Aspartic Acid, Cysteine, Glutamine, Glutamic Acid, Glycine, Isoleucine, Leucine, Methionine, Phenylalanine, Proline, Serine, Threonine, Tryptophan, Tyrosine, Valine and Histidine
  VARIANT 111: note = Arginine or lysine

SEQ ID NO: 6 - protein, 230 aa, synthetic construct; identical to SEQ ID NO: 3
  VARIANT 108..110: note = selected from the group consisting of Valine, Alanine, Glycine, Serine, Threonine, Tyrosine, Asparagine, Aspartic Acid, Glutamine, Glutamic Acid, Methionine and Histidine
  VARIANT 111: note = Arginine or Lysine

SEQ ID NO: 7 - protein, 230 aa, synthetic construct; identical to SEQ ID NO: 3
  VARIANT 108: note = Alanine or Valine
  VARIANT 110: note = Alanine or Valine
  VARIANT 109: note = selected from non-basic amino acids and histidine
  VARIANT 111: note = Arginine or Lysine

SEQ ID NO: 8 - protein, 230 aa, synthetic construct; identical to SEQ ID NO: 3
  VARIANT 109: note = Valine or Serine
  VARIANT 108: note = selected from non-basic amino acids and histidine
  VARIANT 110: note = selected from non-basic amino acids and histidine
  VARIANT 111: note = Arginine or Lysine

SEQ ID NO: 9 - protein, 230 aa, synthetic construct
  VARIANT 108..110: note = selected from non-basic amino acids and histidine
MAPMKEANIRGQGGLAYPGVRTHGTLESVNGPKAGSRGLTSLADTFEHVIEELLDEDQKVRPNEENNKDADLYTSRVMLSSQVPLEPPLLFLLEEYKNYLDAANMSMXXXRHSDPARRGELSVCDSISEWVTAADKKTAVDMSGGTVTVLEKVPVSKGQLKQYFYETKCNPMGYTKEGCRGIDKRHWNSQCRTTQSYVRALTMDSKKRIGWRFIRIDTSCVCTLTIKRGR

SEQ ID NO: 10 - protein, 230 aa, synthetic construct; identical to SEQ ID NO: 9
  VARIANT 108: note = Alanine or Valine
  VARIANT 109: note = Valine or Serine
  VARIANT 110: note = Alanine or Valine

SEQ ID NO: 11 - protein, 5 aa, synthetic construct
MAPMK

SEQ ID NO: 12 - protein, 5 aa, synthetic construct
EANIR

SEQ ID NO: 13 - protein, 11 aa, synthetic construct
GQGGLAYPGVR

SEQ ID NO: 14 - protein, 12 aa, synthetic construct
THGTLESVNGPK

SEQ ID NO: 15 - protein, 4 aa, synthetic construct
AGSR

SEQ ID NO: 16 - protein, 22 aa, synthetic construct
GLTSLADTFEHVIEELLDEDQK

SEQ ID NO: 17 - protein, 7 aa, synthetic construct
PNEENNK

SEQ ID NO: 18 - protein, 8 aa, synthetic construct
DADLYTSR

SEQ ID NO: 19 - protein, 21 aa, synthetic construct
VMLSSQVPLEPPLLFLLEEYK

SEQ ID NO: 20 - protein, 14 aa, synthetic construct
NYLDAANMSMVSAR

SEQ ID NO: 21 - protein, 7 aa, synthetic construct
HSDPARR

SEQ ID NO: 22 - protein, 112 aa, synthetic construct
GELSVCDSISEWVTAADKKTAVDMSGGTVTVLEKVPVSKGQLKQYFYETKCNPMGYTKEGCRGIDKRHWNSQCRTTQSYVRALTMDSKKRIGWRFIRIDTSCVCTLTIKRGR